European Patent Specification EP 3 523 452 B1, published April 15, 2026. Title: Methods for Preparing Oligonucleotides for Detecting a Target Nucleic Acid Molecule in a Sample. Applicant: Seegene, Inc. The sequence listing filed with the application follows.

SEQUENCE LISTING (34 sequences)

SEQ ID NO: 1 - DNA, 2026 bp, Candida albicans
  gene (1)..(2026): PHR1 gene sequence
gaattcatcgacgcctcattcatactaatataataggtgttgcaacatcaaaatcatttcatcgctaatacaaacatccgagattaatcttgtccattggcaatataattaacaccactgccaatacatataaatcaaatcagcattaactaatagtatttattaattacttagaaaagccgggctgcgtttttttgtttcattcatagatttacttatttccatttaacataccaaactacaggttgaagccaaaaaaaaatgtattcattaatcaaatcattggccacatttgccacactcttttcattaactttagccaagtttgaatcgtccaccccaccagttgaagttgttggtaacaaattttatttttccaataatgggtctcagtttttaatcaggggtatcgcctatcagcaagatgccgcgggctcagtttcctccggttacgacgccgatcctaatagaaaatacaatgatcctttagccgatcgtgacgcttgtaaacgtgacgtcaagtatttcaaagaatcaaacaccaatactttgagagtttatgctattgacccagataaggatcatgaagagtgtatgaaaattttcagtgacgctggtatttacattgttgctgatttatcagaaccaactgtatcgattaacagaaacaacccagaatggaacttggatttatacaaacgttatacaaaagtcattgataagatgcaagaatattctaatgttttgggattttttgctggtaacgaagtaactaataatcgttcaaataccgatgcttctgcatttgttaaggctgccattagagatatgaagaaatacatcaaggagtctgattatagacaaattcctgttggttattcatccaatgatgacgaagaaattagagtcgccattgccgattatttctcttgtggttcattagatgatcgtgctgatttctttggtatcaatatgtatgaatggtgtggcaaatcaactttcgaaacctcaggttacaaggacagaactgaagaaatcaagaacttgactatcccagccttcttctccgaatatggatgtaatgctaaccgtccacgtttgttccaagaaattggtaccttgtattccgataagatgactgatgtttggtccggaggtattgtttatatgtattttgaagaggctaacaaatacggtttggttctggttgatggtaattcggtcaagacattatctgactacaacaattacaaatcagaaatgaacaaaataagcccatcccttgcccatacttcaacattatccagttctgacgccagcaagactttgcaatgtccaggaactgctgctagcacttggaaagctgcaactaatttgccaccaactccagatgaaagttactgtgattgtatttccaagtcattagaatgtgttgttgctgacgatgttgataaagaagactatggtgacttgtttggtcaagtttgtggttatatcgattgctcggctatttctgccgatggtagcaaaggtgaatatggtgttgcttccttctgttctgataaagatcgtttgtcatatgtgttgaaccagtattaccttgaccaagacaagaaatccagtgcttgtgatttcaaaggcagtgcttcaatcaatagcaaggctagtgctagtggcagctgcaaagctgttagtggagtagctactggtaaggcatcttcctctggtggaagctccaaatctggatcttcctctgcatctgcttctggatcatcaagcagcagcaccagctctgggtccagctcaagctctggagttaaagcaactcaacaaatgtctatggtcaaattggtttcaattattactattgttactgcatttgttggtggtatgtccgttgttttttaaatcaatgaagactaaccgatatgaagggttctgttgtataggacgaatatatatagtttaataagagttcattatttaaaagttccaatttgaaatcaacttggtacacatatctatt

SEQ ID NO: 2 - DNA, 33 bp, Artificial Sequence
  Probe sequence
gygttgcaacatcaaaatcatttcatcgctaat

SEQ ID NO: 3 - DNA, 34 bp, Artificial Sequence
  Probe sequence
caagttgayttcaaattggaacttttaaataatg

SEQ ID NO: 4 - DNA, 34 bp, Artificial Sequence
  Probe sequence
gttgayttcaaattggaacttttaaataatgawc

SEQ ID NO: 5 - DNA, 33 bp, Artificial Sequence
  Probe sequence
cataccaaactacaggttgragscaaaaaaaaw

SEQ ID NO: 6 - DNA, 30 bp, Artificial Sequence
  Probe sequence
ccaaactacaggttgaagscaaaaaaaawd

SEQ ID NO: 7 - DNA, 31 bp, Artificial Sequence
  Probe sequence
gtattcattaatcaaatcattggyyacattt

SEQ ID NO: 8 - DNA, 29 bp, Artificial Sequence
  Probe sequence
ggyyacatttgccacactcttttcattaa

SEQ ID NO: 9 - DNA, 33 bp, Artificial Sequence
  Probe sequence
gyyacatttgccacactcttttcattaacttta

SEQ ID NO: 10 - DNA, 25 bp, Artificial Sequence
  Primer sequence
tataataggygttgcaacatcaaaa

SEQ ID NO: 11 - DNA, 23 bp, Artificial Sequence
  Primer sequence
aggygttgcaacatcaaaatcat

SEQ ID NO: 12 - DNA, 24 bp, Artificial Sequence
  Primer sequence
acataccaaactacaggttgrags

SEQ ID NO: 13 - DNA, 22 bp, Artificial Sequence
  Primer sequence
caaactacaggttgragscaaa

SEQ ID NO: 14 - DNA, 23 bp, Artificial Sequence
  Primer sequence
tacaggttgragscaaaaaaaaw

SEQ ID NO: 15 - DNA, 22 bp, Artificial Sequence
  Primer sequence
caggttgaagscaaaaaaaawd

SEQ ID NO: 16 - DNA, 21 bp, Artificial Sequence
  Primer sequence
cattaatcaaatcattggyya

SEQ ID NO: 17 - DNA, 18 bp, Artificial Sequence
  Primer sequence
cktccacyccaccarttg

SEQ ID NO: 18 - DNA, 12 bp, Artificial Sequence
  Sequence of tagging portion
gtcccgacgata

SEQ ID NO: 19 - DNA, 28 bp, Artificial Sequence
  Sequence of targeting portion
cattgccgattatttctcttgtggttca

SEQ ID NO: 20 - DNA, 30 bp, Artificial Sequence
  Sequence of targeting portion
gataaatcagcaacaatgtaaataccagcg

SEQ ID NO: 21 - DNA, 29 bp, Artificial Sequence
  Sequence of targeting portion
gtatgaatggtgtggcaaatcaactttcg

SEQ ID NO: 22 - DNA, 29 bp, Artificial Sequence
  Sequence of targeting portion
gacgctggtatttacattgttgctgattt

SEQ ID NO: 23 - DNA, 29 bp, Artificial Sequence
  Sequence of targeting portion
gttaccagcaaaaaatcccaaaacattag

SEQ ID NO: 24 - DNA, 20 bp, Artificial Sequence
  Primer sequence
ttgggattttttgctggtaa

SEQ ID NO: 25 - DNA, 21 bp, Artificial Sequence
  Primer sequence
agttgatttgccacaccattc

SEQ ID NO: 26 - DNA, 23 bp, Artificial Sequence
  Primer sequence
tgagagtttatgctattgaccca

SEQ ID NO: 27 - DNA, 20 bp, Artificial Sequence
  Primer sequence
ccagcaaaaaatcccaaaac

SEQ ID NO: 28 - DNA, 20 bp, Artificial Sequence
  Primer sequence
gccattgccgattatttctc

SEQ ID NO: 29 - DNA, 18 bp, Artificial Sequence
  Primer sequence
tcggagaagaaggctggg

SEQ ID NO: 30 - DNA, 23 bp, Artificial Sequence
  Primer sequence
tgagagtttatgctattgaccca

SEQ ID NO: 31 - DNA, 20 bp, Artificial Sequence
  Primer sequence
ccagcaaaaaatcccaaaac

SEQ ID NO: 32 - DNA, 21 bp, Artificial Sequence
  Primer sequence
cagaaacaacccagaatggaa

SEQ ID NO: 33 - DNA, 20 bp, Artificial Sequence
  Primer sequence
gagaaataatcggcaatggc

SEQ ID NO: 34 - DNA, 38 bp, Artificial Sequence
  CTO sequence
ttttcttttcttttcttttctttttgtatcgtcgggac